European Patent Specification EP 3 883 917 B1, published January 24, 2024. Title: CATIONIC LIPID COMPOUNDS. Applicant: Translate Bio, Inc. DeRosa, Frank Karve, Shrirang Zhang, Yi. The sequence listing filed with the application follows.

SEQUENCE LISTING (4 sequences)

SEQ ID NO: 1 - RNA, 584 nt, Human erythropoietin (EPO) mRNA
  5'UTR (1)..(1)
  3'UTR (584)..(584)
naugggugugcacgaauguccugcuuggcuguggcuccuucucucccugcugucccugccucuuggacucccggugcuuggagcacccccgagacugaucugcgacagcagggugcucgagcgcuaccuccuggaagccaaggaagccgaaaacaucacuacuggcugcgccgaacacugcucccugaacgagaacaucaccgugccggacaccaaggucaacuucuacgcguggaagagaauggaggucggacagcaagccguggaaguguggcagggacuugcgcuccugucggaagccgugcugaggggacaagcccugcucgugaacagcucacagccuugggagccccugcagcugcaugucgacaaggccguguccggacugcgcucacugaccacucugcugagggccuugggugcccagaaagaggcuauuuccccaccggaugcagccucggcagcuccucugcggaccauuacggcggacaccuuucggaagcuguuccgcgucuacagcaauuuccuccgggggaaguugaaacuguauaccggcgaagccugucggacuggcgaucgcugan

SEQ ID NO: 2 - RNA, 1654 nt, Codon-Optimized Firefly Luciferase (FFL) mRNA
  5'UTR (1)..(1)
  3'UTR (1654)..(1654)
nauggaagaugccaaaaacauuaagaagggcccagcgccauucuacccacucgaagacgggaccgccggcgagcagcugcacaaagccaugaagcgcuacgcccuggugcccggcaccaucgccuuuaccgacgcacauaucgagguggacauuaccuacgccgaguacuucgagaugagcguucggcuggcagaagcuaugaagcgcuaugggcugaauacaaaccaucggaucguggugugcagcgagaauagcuugcaguucuucaugcccguguugggugcccuguucaucgguguggcuguggccccagcuaacgacaucuacaacgagcgcgagcugcugaacagcaugggcaucagccagcccaccgucguauucgugagcaagaaagggcugcaaaagauccucaacgugcaaaagaagcuaccgaucauacaaaagaucaucaucauggauagcaagaccgacuaccagggcuuccaaagcauguacaccuucgugacuucccauuugccacccggcuucaacgaguacgacuucgugcccgagagcuucgaccgggacaaaaccaucgcccugaucaugaacaguaguggcaguaccggauugcccaagggcguagcccuaccgcaccgcaccgcuuguguccgauucagucaugcccgcgaccccaucuucggcaaccagaucauccccgacaccgcuauccucagcguggugccauuucaccacggcuucggcauguucaccacgcugggcuacuugaucugcggcuuucgggucgugcucauguaccgcuucgaggaggagcuauucuugcgcagcuugcaagacuauaagauucaaucugcccugcuggugcccacacuauuuagcuucuucgcuaagagcacucucaucgacaaguacgaccuaagcaacuugcacgagaucgccagcggcggggcgccgcucagcaaggagguaggugaggccguggccaaacgcuuccaccuaccaggcauccgccagggcuacggccugacagaaacaaccagcgccauucugaucacccccgaaggggacgacaagccuggcgcaguaggcaagguggugcccuucuucgaggcuaaggugguggacuuggacaccgguaagacacugggugugaaccagcgcggcgagcugugcguccguggccccaugaucaugagcggcuacguuaacaaccccgaggcuacaaacgcucucaucgacaaggacggcuggcugcacagcggcgacaucgccuacugggacgaggacgagcacuucuucaucguggaccggcugaagagccugaucaaauacaagggcuaccagguagccccagccgaacuggagagcauccugcugcaacaccccaacaucuucgacgccggggucgccggccugcccgacgacgaugccggcgagcugcccgccgcagucgucgugcuggaacacgguaaaaccaugaccgagaaggagaucguggacuauguggccagccagguuacaaccgccaagaagcugcgcggugguguuguguucguggacgaggugccuaaaggacugaccggcaaguuggacgcccgcaagauccgcgagauucucauuaaggccaagaagggcggcaagaucgccguguan

SEQ ID NO: 3 - RNA, 140 nt, 5' UTR
ggacagaucgccuggagacgccauccacgcuguuuugaccuccauagaagacaccgggaccgauccagccuccgcggccgggaacggugcauuggaacgcggauuccccgugccaagagugacucaccguccuugacacg

SEQ ID NO: 4 - RNA, 100 nt, 3'UTR
cggguggcaucccugugaccccuccccagugccucuccuggcccuggaaguugccacuccagugcccaccagccuuguccuaauaaaauuaaguugcauc